European Patent Specification EP 3 898 659 B1, published September 16, 2026. Title: Novel FOLR1 specific binding proteins for cancer diagnosis and treatment. Applicant: Navigo Proteins GmbH. The sequence listing filed with the application follows.

SEQUENCE LISTING (73 sequences)

SEQ ID NO: 1 - protein, 76 aa, Artificial Sequence
  197556a
MQIFVKTLEEKYIALEVEPCDTIENVKAKVQDKEGIPPDQQELLWYGEQLEDGRTLSDYNILGGAVLKLQLRLRAA

SEQ ID NO: 2 - protein, 76 aa, Artificial Sequence
  197556b
MQIFVKTLEEKYIALEVEPSDTIENVKAKVQDKEGIPPDQQELLWYGEQLEDGRTLSDYNILGGAVLKLQLRLRAA

SEQ ID NO: 3 - protein, 76 aa, Artificial Sequence
  197251
MQIFVKTLEEKYITLEVEPSDTIENVKAKVQGKEGIPPDQQELLWYGEQLEGGRTLSDYNILGGAVLKLQLRLRAA

SEQ ID NO: 4 - protein, 76 aa, Artificial Sequence
  196962
MQIFVKTLEEKYTTLEVEPSDTIENVKARIQDKEGIPPDQQKLLWYGEQLEDGRTLSDYNILGGAVLKLQLRLRAA

SEQ ID NO: 5 - protein, 76 aa, Artificial Sequence
  197525
MQIFVKTLEEKYITLEVEPSDTIENVKARVQDKEGIPPDQQKLLWYGEQLEDGRTLSDYNILGGAVLKLQLRLRAA

SEQ ID NO: 6 - protein, 76 aa, Artificial Sequence
  187731
MQIFVKTLEEKYITLEVEPSDTIENVKAKIQDKEGIPPDQQKLLWYGKQLEDGRTLSDYNILGGAVLKLQLRLRAA

SEQ ID NO: 7 - protein, 76 aa, Artificial Sequence
  197132
MQIFVKTLEEKYITLEVEPSDTIENVKAKIQDKEGIPPDQQKLLWYGKQLEDGRTLSDHNILGGAVLKLQLRLRAA

SEQ ID NO: 8 - protein, 76 aa, Artificial Sequence
  197340
MQIFVKTLEERYITLEVEPSDTIENVKAKIQDKEGIPPDQQKLLWYGERLEDGRTLSNYNILGGAVLKLQLRLRAA

SEQ ID NO: 9 - protein, 76 aa, Artificial Sequence
  196920
MQIFVKTLEERYITLEVEPSDTIENVKAKIQGKEGIPPDQQKLLWYGEQLKDGRTLSDYSILGGAVLKLQLRLRAA

SEQ ID NO: 10 - protein, 76 aa, Artificial Sequence
  197103
MQIFVKTLEEKYITLEVEPSDTTEDVKAKIQDKEGIPPDQQKLLWYGEQLEDGRTLSDYNILGGAVLKLQPRLRAA

SEQ ID NO: 11 - protein, 76 aa, Artificial Sequence
  197032
MQIFVKTLEEKYITLEVEPSDTIENVKAKIQDKEGIPPDQQKLLRYGKQLEDGRTLSDYNILGGAVLKLQPRLRAA

SEQ ID NO: 12 - protein, 76 aa, Artificial Sequence
  196964
MQIFVKTLEEKYITLEVEPSDTIENVKAKLQDKEGIPPDQQKLLWYGKQLEDGRTLSDYTILGGAVLKLQLRLRAA

SEQ ID NO: 13 - protein, 76 aa, Artificial Sequence
  197312
MQIFVKTLEEKYIPLEVEPSDTIENVKATIQDKEGIPPDQQKLLWYGKQLDDGRTLSDYNILGGAVLKLQLRLRAA

SEQ ID NO: 14 - protein, 76 aa, Artificial Sequence
  196868
MQIFVKTLEEKYITLEVEPSDTIENVKAKIQDKEGIPPDQQKLLWYGKQLEDGRTLSDYTILGGAVLKLQLRLRAA

SEQ ID NO: 15 - protein, 76 aa, Artificial Sequence
  197044
MQIFVKTLEEKYITLEVEPGDTIENVKAEIQDKEGIPPDQQKLLWYGKQLEDGRTLSDYNILGGAVLKLQPRLRAA

SEQ ID NO: 16 - protein, 76 aa, Artificial Sequence
  197230
MQIFVKTLEEKYITLEVEPSDTIENVKAEIQGREGIPPDQQKLLWYGKQLEDGRTLSDYNILGGAVLKLQLRLRAA

SEQ ID NO: 17 - protein, 76 aa, Artificial Sequence
  197383
MQIFVKTLEEKYITLEVEPSDTIENVKAKIQNKEGIPPDQQKLLWYGEQLEDGRTLSDYNILGDAVLKLQLRLRAA

SEQ ID NO: 18 - protein, 76 aa, Artificial Sequence
  196934
MQIFVKTLEERYITLEVEPSDTIGNVKAKIQDKEGIPPDQQKLLWYGEQLEDGRTLSDYNILGDAVLKLQLRLRAA

SEQ ID NO: 19 - protein, 76 aa, Artificial Sequence
  197126
MQIFVKTLEEKYITLEVEPSDTIANVKAKIQDKEGIPPDQQKLLWYGKQLEDGRTLSDYNILGGAVLKLPLRLRAA

SEQ ID NO: 20 - protein, 76 aa, Artificial Sequence
  197014
MQIFVKTLEEKYIPLEVEPSDTIENVKAKIQDKEGIPPDQQKLLWYGKQLEDGRTLSDYNILGGAVLKLPLRLRAA

SEQ ID NO: 21 - protein, 76 aa, Artificial Sequence
  196888
MQIFVKTLEEKYITLEVEPSDTIENVKAKIQDKEGIPPDQQKLLWYGKQLEDGRTLSDYNILGGAVLKLPLRLRAA

SEQ ID NO: 22 - protein, 76 aa, Artificial Sequence
  197106
MQIFVKTLEEKYITLEVEPSDTIENVKAKIQDQAGIPPDQQKLLWYGKQLEDGRTLSDYNILGGAVLKLPLRLRAA

SEQ ID NO: 23 - protein, 76 aa, Artificial Sequence
  197252
MQIFVKTLEEKYITLEVEPSDTVENVKAKIRDKEGIPPDQQKLLWYGKQLEGGRTLSDYNILGGAVLKLQLGLRAA

SEQ ID NO: 24 - protein, 76 aa, Artificial Sequence
  189864
MQIFVVTRLYKEITLEVEPSDTIENVKAKIQDKEGIPPDQQYLYWDGKQLEDGRTLSDYNIRFGDHLDLTLGLRAA

SEQ ID NO: 25 - protein, 76 aa, Artificial Sequence
  189872
MQIFVVTRLYKEITLEVEPSDTIENVKAKIQDKEGIPPDQQYLYGDGKQLEDGRTLSDYNIRFGDHLDLTLGLRAA

SEQ ID NO: 26 - protein, 76 aa, Artificial Sequence
  181919
MQIFVVTRLYKEITLEVEPSDTIENVKAKIQDKEGIPPDQQYLYWDGKQLEDGRTLSDYNIRFGYHLDLTLGLRAA

SEQ ID NO: 27 - protein, 76 aa, Artificial Sequence
  189853
MQIFVVTRLYKETALEVEPSDTIENVKAKIQDKEGIPPDQQYLYWDGKQLEDGRTLSDYNIRFGYHLDLTLGLRAA

SEQ ID NO: 28 - protein, 76 aa, Artificial Sequence
  187770
MQIFVVTESYKWITLEVEPSDTIENVKAKIQDKEGIPPDQQQLVWDGKQLEDGRTLSDYNIDLGGYLPLWLYLRAA

SEQ ID NO: 29 - protein, 76 aa, Artificial Sequence
  187803
MQIFVQTYNIKDITLEVEPSDTIENVKAKIQDKEGIPPDQQMLFWSGKQLEDGRTLSDYNIIAYMTLTLHLKLRAA

SEQ ID NO: 30 - protein, 168 aa, Artificial Sequence
  199490
MQIFVKTLEEKYIALEVEPSDTIENVKAKVQDKEGIPPDQQELLWYGEQLEDGRTLSDYNILGGAVLKLQLRLRAAGGSGGGSGGGSGGGSGMQIFVKTLEEKYIALEVEPSDTIENVKAKVQDKEGIPPDQQELLWYGEQLEDGRTLSDYNILGGAVLKLQLRLRAA

SEQ ID NO: 31 - protein, 152 aa, Artificial Sequence
  199489 dimer of SEQ ID NO: 2
MQIFVKTLEEKYIALEVEPSDTIENVKAKVQDKEGIPPDQQELLWYGEQLEDGRTLSDYNILGGAVLKLQLRLRAAMQIFVKTLEEKYIALEVEPSDTIENVKAKVQDKEGIPPDQQELLWYGEQLEDGRTLSDYNILGGAVLKLQLRLRAA

SEQ ID NO: 32 - protein, 168 aa, Artificial Sequence
  199484 homodimer of SEQ ID NO 4
MQIFVKTLEEKYTTLEVEPSDTIENVKARIQDKEGIPPDQQKLLWYGEQLEDGRTLSDYNILGGAVLKLQLRLRAAGGSGGGSGGGSGGGSGMQIFVKTLEEKYTTLEVEPSDTIENVKARIQDKEGIPPDQQKLLWYGEQLEDGRTLSDYNILGGAVLKLQLRLRAA

SEQ ID NO: 33 - protein, 152 aa, Artificial Sequence
  199483 homodimer of SEQ ID NO: 4
MQIFVKTLEEKYTTLEVEPSDTIENVKARIQDKEGIPPDQQKLLWYGEQLEDGRTLSDYNILGGAVLKLQLRLRAAMQIFVKTLEEKYTTLEVEPSDTIENVKARIQDKEGIPPDQQKLLWYGEQLEDGRTLSDYNILGGAVLKLQLRLRAA

SEQ ID NO: 34 - protein, 168 aa, Artificial Sequence
  199488 homo-dimer of SEQ ID NO: 5
MQIFVKTLEEKYITLEVEPSDTIENVKARVQDKEGIPPDQQKLLWYGEQLEDGRTLSDYNILGGAVLKLQLRLRAAGGSGGGSGGGSGGGSGMQIFVKTLEEKYITLEVEPSDTIENVKARVQDKEGIPPDQQKLLWYGEQLEDGRTLSDYNILGGAVLKLQLRLRAA

SEQ ID NO: 35 - protein, 152 aa, Artificial Sequence
  199487 homo-dimer of SEQ ID NO: 5
MQIFVKTLEEKYITLEVEPSDTIENVKARVQDKEGIPPDQQKLLWYGEQLEDGRTLSDYNILGGAVLKLQLRLRAAMQIFVKTLEEKYITLEVEPSDTIENVKARVQDKEGIPPDQQKLLWYGEQLEDGRTLSDYNILGGAVLKLQLRLRAA

SEQ ID NO: 36 - protein, 168 aa, Artificial Sequence
  199478 homodimer of SEQ ID NO: 6
MQIFVKTLEEKYITLEVEPSDTIENVKAKIQDKEGIPPDQQKLLWYGKQLEDGRTLSDYNILGGAVLKLQLRLRAAGGSGGGSGGGSGGGSGMQIFVKTLEEKYITLEVEPSDTIENVKAKIQDKEGIPPDQQKLLWYGKQLEDGRTLSDYNILGGAVLKLQLRLRAA

SEQ ID NO: 37 - protein, 152 aa, Artificial Sequence
  199477 homodimer of SEQ ID NO: 6
MQIFVKTLEEKYITLEVEPSDTIENVKAKIQDKEGIPPDQQKLLWYGKQLEDGRTLSDYNILGGAVLKLQLRLRAAMQIFVKTLEEKYITLEVEPSDTIENVKAKIQDKEGIPPDQQKLLWYGKQLEDGRTLSDYNILGGAVLKLQLRLRAA

SEQ ID NO: 38 - protein, 152 aa, Artificial Sequence
  199479 homodimer of SEQ ID NO 18
MQIFVKTLEERYITLEVEPSDTIGNVKAKIQDKEGIPPDQQKLLWYGEQLEDGRTLSDYNILGDAVLKLQLRLRAAMQIFVKTLEERYITLEVEPSDTIGNVKAKIQDKEGIPPDQQKLLWYGEQLEDGRTLSDYNILGDAVLKLQLRLRAA

SEQ ID NO: 39 - protein, 162 aa, Artificial Sequence
  199480 homodimer of SEQ ID NO. 18
MQIFVKTLEERYITLEVEPSDTIGNVKAKIQDKEGIPPDQQKLLWYGEQLEDGRTLSDYNILGDAVLKLQLRLRAAGGSGGGSGGGMQIFVKTLEERYITLEVEPSDTIGNVKAKIQDKEGIPPDQQKLLWYGEQLEDGRTLSDYNILGDAVLKLQLRLRAA

SEQ ID NO: 40 - protein, 168 aa, Artificial Sequence
  199481 homodimer of SEQ ID NO 18
MQIFVKTLEERYITLEVEPSDTIGNVKAKIQDKEGIPPDQQKLLWYGEQLEDGRTLSDYNILGDAVLKLQLRLRAAGGSGGGSGGGSGGGSGMQIFVKTLEERYITLEVEPSDTIGNVKAKIQDKEGIPPDQQKLLWYGEQLEDGRTLSDYNILGDAVLKLQLRLRAA

SEQ ID NO: 41 - protein, 172 aa, Artificial Sequence
  199482 homodimer of SEQ ID NO 18
MQIFVKTLEERYITLEVEPSDTIGNVKAKIQDKEGIPPDQQKLLWYGEQLEDGRTLSDYNILGDAVLKLQLRLRAAGGSGGGSGGGSGGGSGGGSGMQIFVKTLEERYITLEVEPSDTIGNVKAKIQDKEGIPPDQQKLLWYGEQLEDGRTLSDYNILGDAVLKLQLRLRAA

SEQ ID NO: 42 - protein, 168 aa, Artificial Sequence
  199486 homodimer of SEQ ID NO 20
MQIFVKTLEEKYIPLEVEPSDTIENVKAKIQDKEGIPPDQQKLLWYGKQLEDGRTLSDYNILGGAVLKLPLRLRAAGGSGGGSGGGSGGGSGMQIFVKTLEEKYIPLEVEPSDTIENVKAKIQDKEGIPPDQQKLLWYGKQLEDGRTLSDYNILGGAVLKLPLRLRAA

SEQ ID NO: 43 - protein, 152 aa, Artificial Sequence
  199485 homodimer of SEQ ID NO: 20
MQIFVKTLEEKYIPLEVEPSDTIENVKAKIQDKEGIPPDQQKLLWYGKQLEDGRTLSDYNILGGAVLKLPLRLRAAMQIFVKTLEEKYIPLEVEPSDTIENVKAKIQDKEGIPPDQQKLLWYGKQLEDGRTLSDYNILGGAVLKLPLRLRAA

SEQ ID NO: 44 - protein, 171 aa, Artificial Sequence
  202521 (199490) homodimer of SEQ ID NO 2 with C-terminal SAC but no Streptag
MQIFVKTLEEKYIALEVEPSDTIENVKAKVQDKEGIPPDQQELLWYGEQLEDGRTLSDYNILGGAVLKLQLRLRAAGGSGGGSGGGSGGGSGMQIFVKTLEEKYIALEVEPSDTIENVKAKVQDKEGIPPDQQELLWYGEQLEDGRTLSDYNILGGAVLKLQLRLRAASAC

SEQ ID NO: 45 - protein, 181 aa, Artificial Sequence
  199490 (homodimer of SEQ ID NO 2) with c-terminal SAC and Streptag
MQIFVKTLEEKYIALEVEPSDTIENVKAKVQDKEGIPPDQQELLWYGEQLEDGRTLSDYNILGGAVLKLQLRLRAAGGSGGGSGGGSGGGSGMQIFVKTLEEKYIALEVEPSDTIENVKAKVQDKEGIPPDQQELLWYGEQLEDGRTLSDYNILGGAVLKLQLRLRAASACASWSHPQFEK

SEQ ID NO: 46 - protein, 76 aa, Artificial Sequence
  ubiquitin
MQIFVKTLTGKTITLEVEPSDTIENVKAKIQDKEGIPPDQQRLIWAGKQLEDGRTLSDYNIQKESTLHLVLRLRAA

SEQ ID NO: 47 - protein, 9 aa, Artificial Sequence
  motif 62-70
LGGAVLKLQ

SEQ ID NO: 48 - protein, 9 aa, Artificial Sequence
  motif 62-70
LGDAVLKLQ

SEQ ID NO: 49 - protein, 9 aa, Artificial Sequence
  motif 62-70
LGGAVLKLP

SEQ ID NO: 50 - protein, 9 aa, Artificial Sequence
  motif 62-70
RFGDHLDLT

SEQ ID NO: 51 - protein, 9 aa, Artificial Sequence
  motif 62-70
RFGYHLDLT

SEQ ID NO: 52 - protein, 9 aa, Artificial Sequence
  motif 62-70
DLGGYLPLW

SEQ ID NO: 53 - protein, 9 aa, Artificial Sequence
  motif 62-70
IAYMTLTLH

SEQ ID NO: 54 - protein, 5 aa, Artificial Sequence
  motif 42-46
ELLWY

SEQ ID NO: 55 - protein, 5 aa, Artificial Sequence
  motif 42-46
KLLWY

SEQ ID NO: 56 - protein, 5 aa, Artificial Sequence
  motif 42-46
KLLRY

SEQ ID NO: 57 - protein, 5 aa, Artificial Sequence
  motif 42-46
YLYWD

SEQ ID NO: 58 - protein, 5 aa, Artificial Sequence
  motif 42-46
YLYGD

SEQ ID NO: 59 - protein, 5 aa, Artificial Sequence
  motif 42-46
QLVWD

SEQ ID NO: 60 - protein, 5 aa, Artificial Sequence
  motif 42-46
MLFWS

SEQ ID NO: 61 - protein, 4 aa, Artificial Sequence
  motif 9-12
EEKY

SEQ ID NO: 62 - protein, 4 aa, Artificial Sequence
  motif 9-12
EERY

SEQ ID NO: 63 - protein, 4 aa, Artificial Sequence
  motif 9-12
EQKY

SEQ ID NO: 64 - protein, 4 aa, Artificial Sequence
  motif 9-12
LYKE

SEQ ID NO: 65 - protein, 4 aa, Artificial Sequence
  motif 9-12
SYKW

SEQ ID NO: 66 - protein, 4 aa, Artificial Sequence
  motif 9-12
NIKD

SEQ ID NO: 67 - protein, 16 aa, Artificial Sequence
  linker
GGSGGGSGGGSGGGSG

SEQ ID NO: 68 - protein, 10 aa, Artificial Sequence
  c-terminal sequence (StrepTaq)
ASWSHPQFEK

SEQ ID NO: 69 - protein, 76 aa, Artificial Sequence
  Affilin 197103 E10Q
MQIFVKTLEQKYITLEVEPSDTTEDVKAKIQDKEGIPPDQQKLLWYGEQLEDGRTLSDYNILGGAVLKLQPRLRAA

SEQ ID NO: 70 - protein, 76 aa, Artificial Sequence
  Affilin 197312 E10Q
MQIFVKTLEQKYIPLEVEPSDTIENVKATIQDKEGIPPDQQKLLWYGKQLDDGRTLSDYNILGGAVLKLQLRLRAA

SEQ ID NO: 71 - protein, 76 aa, Artificial Sequence
  Affilin 197014 E10Q
MQIFVKTLEQKYIPLEVEPSDTIENVKAKIQDKEGIPPDQQKLLWYGKQLEDGRTLSDYNILGGAVLKLPLRLRAA

SEQ ID NO: 72 - protein, 168 aa, Artificial Sequence
  Affilin 199486 E10Q
MQIFVKTLEQKYIPLEVEPSDTIENVKAKIQDKEGIPPDQQKLLWYGKQLEDGRTLSDYNILGGAVLKLPLRLRAAGGSGGGSGGGSGGGSGMQIFVKTLEQKYIPLEVEPSDTIENVKAKIQDKEGIPPDQQKLLWYGKQLEDGRTLSDYNILGGAVLKLPLRLRAA

SEQ ID NO: 73 - protein, 152 aa, Artificial Sequence
  Affilin 199485 E10Q
MQIFVKTLEQKYIPLEVEPSDTIENVKAKIQDKEGIPPDQQKLLWYGKQLEDGRTLSDYNILGGAVLKLPLRLRAAMQIFVKTLEQKYIPLEVEPSDTIENVKAKIQDKEGIPPDQQKLLWYGKQLEDGRTLSDYNILGGAVLKLPLRLRAA